European Patent Application EP 4 162 951 A1, published April 12, 2023. Title: PHARMACEUTICAL COMPOSITION OF ENZYMES AND VIRUSES AND APPLICATION THEREOF. Applicant: Shanghai Bao Pharmaceuticals Co., Ltd. The sequence listing filed with the application follows.

SEQUENCE LISTING (47 sequences)

SEQ ID NO: 1 - protein, 339 aa, Artificial sequence
  IdeS
MRKRCYSTSAAVLAAVTLFVLSVDRGVIADSFSANQEIRYSEVTPYHVTSVWTKGVTPPANFTQGEDVFHAPYVANQGWYDITKTFNGKDDLLCGAATAGNMLHWWFDQNKDQIKRYLEEHPEKQKINFNGEQMFDVKEAIDTKNHQLDSKLFEYFKEKAFPYLSTKHLGVFPDHVIDMFINGYRLSLTNHGPTPVKEGSKDPRGGIFDAVFTRGDQSKLLTSRHDFKEKNLKEISDLIKKELTEGKALGLSHTYANVRINHVINLWGADFDSNGNLKAIYVTDSDSNASIGMKKYFVGVNSAGKVAISAKEIKEDNIGAQVLGLFTLSTGQDSWNQTN

SEQ ID NO: 2 - protein, 349 aa, Artificial sequence
  IdeZ
MKTIAYPNKPHSLSAGLLTAIAIFSLASSNITYADDYQRNATEAYAKEVPHQITSVWTKGVTPLTPEQFRYNNEDVIHAPYLAHQGWYDITKAFDGKDNLLCGAATAGNMLHWWFDQNKTEIEAYLSKHPEKQKIIFNNQELFDLKAAIDTKDSQTNSQLFNYFRDKAFPNLSARQLGVMPDLVLDMFINGYYLNVFKTQSTDVNRPYQDKDKRGGIFDAVFTRGDQTTLLTARHDLKNKGLNDISTIIKQELTEGRALALSHTYANVSISHVINLWGADFNAEGNLEAIYVTDSDANASIGMKKYFVGINAHGHVAISAKKIEGENIGAQVLGLFTLSSGKDIWQKLS

SEQ ID NO: 3 - protein, 392 aa, Artificial sequence
  IdeZ2
MMKKQSFTHSRKPKFGMRKLSIGLASCMLGMMFLTTSHVSGEVVEVWPYGQDPNDKIEVLSQSEYSEYLQRLHDVEDFQAEKKKEGVVRTQWLEGVNVTDHDFRKITDGGSVYYATPLLNDRGYYDINKNFNQDSDKCAAAVAVNMFHYWLDRNKDNVAKFLSQSPDHGFVEGEPTFNLVDFQYTYASPYEEGGYRDNSKLFDFISKAFNKPLWANKLLDAYINGYGYIDRYVKNTPHSGQNNSKFNFFKKVFDGKLLTDIQQIFDYYTLSSELREALDTGKAIGLAYGPGDLRRSLGHIISVWGADINEDGNVVAIYVTDSDDKKLTIGNKKDRIGLKRYKLYSDNVGRARLTAYATENQQTGGEVRGIETLDMATQDWADYFSRTDEAEQ

SEQ ID NO: 4 - protein, 349 aa, Artificial sequence
  IdeE
MKTIAYPNKPHSLSAGLLTAIAIFSLASSNITYADDYQRNATEAYAKEVPHQITSVWTKGVTPLTPEQFRYNNEDVIHAPYLAHQGWYDITKAFDGKDNLLCGAATAGNMLHWWFDQNKTEIEAYLSKHPEKQKIIFNNQELFDLKAAIDTKDSQTNSQLFNYFRDKAFPNLSARQLGVMPDLVLDMFINGYYLNVFKTQSTDVNRPYQDKDKRGGIFDAVFTRGDQTTLLTARHDLKNKGLNDISTIIKQELTEGRALALSHTYANVSISHVINLWGADFNAEGNLEAIYVTDSDANASIGMKKYFVGINAHRHVAISAKKIEGENIGAQVLGLFTLSSGKDIWQKLS

SEQ ID NO: 5 - protein, 385 aa, Artificial sequence
  IdeE2
MMKKQSFTHSRKPKFGMRKLSIGLASCMLGMMFLTTGHVSGEVVEVWPNGQNPNGKIEILSQTEHSEHLQKLRDIEDFQAQKQADHVRYTKWLDGVTVDEHEFRKIKEYDTEYYVTPLLSGKGYYDINKDFNQDSDKCAAAVAANMFHYWFDRNRDSINRFLSQSPGENGVIKLENEKTIEVSKFLETYRSDGDYLDKSPFFDLISNSFKGPVWANKLLDAYINGYGYIHKFAKNTPHSKNNNSKFNFFKKVFDGNLLTDIHQIFDYNTFSDKLSEALYTGKAIGLAYGPGDLRRSLGHIISVWGADLDDQNRVVAIYVTDSDDKKLTIGNERVGLKRYKVSSDDQGRARLTTRDKDNTGGEIRSIETLDMGTQEWADYFNKTEK

SEQ ID NO: 6 - protein, 372 aa, Artificial sequence
  IdeP
MNKKNSKGLPRYFRISARTLLLGALLSGGLLSVPEKAHADNRSASTISVSIDSNQNETNLVTAENVQTANLSDPDTKVNTVWTAGMSELDTKQFTPHPDGFLHYPYQSNQGWYNITKSFNGRDNLLCAAATAGNMLHWWFDQNKEQIDRYLKEHPEKANISFRGENFLSIKELINTKGKQKDSALFTYFQEKAFPDISRRNTGLIVDRVLDMFINGYYLSINDLSETNTSNTRKDNRGGVFDHVFGRGDSHKKLTSRYELQDQSIEEIGQLIRRELEAGKALAISYTYASIGMAHVVNLWGADFDQAGQLVAIYVADSDNSTDVGMKKYYVGKNKEGHVAISAQKVEGDVLGSRLLRLGSLSSGKDMWPAQY

SEQ ID NO: 7 - protein, 310 aa, Artificial sequence
  IgG-degrading enzyme mutant
DSFSANQEIRYSEVTPYHVTSVWTKGVTPPANFTQGEDVFHAPYVANQGWYDITKTFNGKDDLLCGAATAGNMLHWWFDQNKDQIKRYLEEHPEKQKINFRGEQMFDVKEAIDTKNHQLDSKLFEYFKEKAFPYLSTKHLGVFPDHVIDMFINGYRLSLTNHGPTPVKEGSKDPRGGIFDAVFTRGDQSKLLTSRHDFKEKNLKEISDLIKKELTEGKALGLSHTYANVRINHVINLWGADFDSNGNLKAIYVTDSDSNASIGMKKYFVGVNSAGKVAISAKEIKEDNIGAQVLGLFTLSTGQDSWNQTN

SEQ ID NO: 8 - protein, 310 aa, Artificial sequence
  IgG-degrading enzyme mutant
DSFSANQEIRYSEVTPYHVTSVWTKGVTPPANFTQGEDVFHAPYVANQGWYDITKTFNGKDDLLCGAATAGNMLHWWFDQNKDQIKRYLEEHPEKQKINFKGEQMFDVKEAIDTKNHQLDSKLFEYFKEKAFPYLSTKHLGVFPDHVIDMFINGYRLSLTNHGPTPVKRGSKDPRGGIFDAVFTRGNQSKLLTSRHDFKEKNLKEISDLIKKELTEGKALGLSHTYANVRINHVINLWGADFDSNGNLKAIYVTDSDSNASIGMKKYFVGVNSAGKVAISAKEIKEDNIGAQVLGLFTLSTGQDSWNQTN

SEQ ID NO: 9 - protein, 310 aa, Artificial sequence
  IgG-degrading enzyme mutant
DSFSANQEIRYSEVTPYHVTSVWTKGVTPPANFTQGEDVFHAPYVANQGWYDITKTFNGKDDLLCGAATAGNMLHWWFDQNKDQIKRYLEEHPEKQKINFRGEQMFDVKEAIDTKNHQLDSKLFEYFKEKAFPYLSTKHLGVFPDHVIDMFINGYRLSLTNHGPTPVKKGSKDPRGGIFDAVFTRGNQSKLLTSRHDFKEKNLKEISDLIKKELTEGKALGLSHTYANVRINHVINLWGADFDSNGNLKAIYVTDSDSNASIGMKKYFVGVNKAGKVAISAKEIKEDNIGAQVLGLFTLSTGQDSWNQTN

SEQ ID NO: 10 - protein, 310 aa, Artificial sequence
  IgG-degrading enzyme mutant
DSFSANQEIRYSEVTPYHVTSVWTKGVTPPANFTQGEDVFHAPYVANQGWYDITKTFNGKDDLLCGAATAGNMLHWWFDQNKDQIKRYLREHPEKQKINFNGEQMFDVKEAIDTKNHQLDSKLFEYFKEKAFPYLSTKHLGVFPDHVIDMFINGYRLSLTNHGPTPVKEGSKDPRGGIFDAVFTRGNQSKLLTSRHDFKEKNLKEISDLIKKELDEGKALGLSHTYANVRINHVINLWGADFDSNGNLKAIYVTDSDSNASIGMKKYFVGVNSAGKVAISAKEIKEDNIGAQVLGLFTLSTGQDSWNQTN

SEQ ID NO: 11 - protein, 310 aa, Artificial sequence
  IgG-degrading enzyme mutant
DSFSANQEIRYSEVTPYHVTSVWTKGVTPPANFTQGEDVFHAPYVANQGWYDITKTFNGKDDLLCGAATAGNMLHWWFDQNKDQIKRYLKEHPEKQKINFNGEQMFDVKEAIRTKNHQLDSKLFEYFKEKAFPYLSTKHLGVFPDHVIDMFINGYRLSLTNHGPTPVKEGSKDPRGGIFDAVFTRGNQSKLLTSRHDFKEKNLKEISDLIKKELEEGKALGLSHTYANVRINHVINLWGADFDSNGNLKAIYVTDSDSNASIGMKKYFVGVNKAGKVAISAKEIKEDNIGAQVLGLFTLSTGQDSWNQTN

SEQ ID NO: 12 - protein, 310 aa, Artificial sequence
  IgG-degrading enzyme mutant
DSFSANQEIRYSEVTPYHVTSVWTKGVTPPANFTQGEDVFHAPYVANQGWYDITKTFNGKDDLLCGAATAGNMLHWWFDQNKDQIERYLEEHPEKQKINFNGEQMFDVKEAIDTKNHQLDSKLFEYFKEKAFPYLSTKHLGVFPDHVIDMFINGYRLSLTNHGPTPVKEGSKDPRGGIFDAVFTRGNQSKLLTSRHDFKEKNLKEISDLIKEELTKGKALGLSHTYANVRINHVINLWGADFDSNGNLKAIYVTDSDSNASIGMKKYFVGVNSAGKVAISAKEIKEKNIGAQVLGLFTLSTGQKSWNQTN

SEQ ID NO: 13 - protein, 310 aa, Artificial sequence
  IgG-degrading enzyme mutant
DSFSANQEIRYSEVTPYHVTSVWTKGVTPPANFTQGEDVFHAPYVANQGWYDITKTFNGKDDLLCGAATAGNMLHWWFDQNKDQIKRYLKEHPEKQKINFRGEQMFDVKEAIRTKNHQLDSKLFEYFKEKAFPYLSTKHLGVFPDHVIDMFINGYRLSLTNHGPTPVKEGSKDPRGGIFDAVFTRGNQSKLLTSRHDFKEKNLKEISDLIKSELENGKALGLSHTYANVRINHVINLWGADFDSNGNLKAIYVTDSDSNASIGMKKYFVGVNKAGKVAISAKEIKEDNIGAQVLGLFTLSTGQDSWNQTN

SEQ ID NO: 14 - protein, 310 aa, Artificial sequence
  IgG-degrading enzyme mutant
DSFSANQEIRYSEVTPYHVTSVWTKGVTPPANFTQGEDVFHAPYVANQGWYDITKTFNGKDDLLCGAATAGNMLHWWFDQNKDQIKRYLKEHPEKQKINFRGEQMFDVKEAIRTKNHQLDSKLFEYFKEKAFPYLSTKHLGVFPDHVIDMFINGYRLSLTNHGPTPVKKGSKDPRGGIFDAVFTRGNQSKLLTSRHDFKEKNLKEISDLIKKELEEGKALGLSHTYANVRINHVINLWGADFDSNGNLKAIYVTDSDSNASIGMKKYFVGVNSAGKVAISAKEIKEDNIGAQVLGLFTLSTGQDSWNQTN

SEQ ID NO: 15 - protein, 310 aa, Artificial sequence
  IgG-degrading enzyme mutant
DSFSANQEIRYSEVTPYHVTSVWTKGVTPPANFTQGEDVFHAPYVANQGWYDITKTFNGKDDLLCGAATAGNMLHWWFDQNKDQIERYLEEHPEKQKINFRGEQMFDVKEAIDTKNHQLDSKLFEYFKEKAFPYLSTKHLGVFPDHVIDMFINGYRLSLTNHGPTPVKKGSKDPRGGIFDAVFTRGNQSKLLTSRHDFKEKNLKEISDLIKEELTKGKALGLSHTYANVRINHVINLWGADFDSNGNLKAIYVTDSDSNASIGMKKYFVGVNSAGKVAISAKEIKEDNIGAQVLGLFTLSTGQKSWNQTN

SEQ ID NO: 16 - protein, 306 aa, Artificial sequence
  IgG-degrading enzyme mutant
DSFSANQEIRYSEVTPYHVTSVWTKGVTPPANFTQGEDVFHAPYVANQGWYDITKTFNGKDDLLCGAATAGNMLHWWFDQNKDQIKRYLEEHPEKQKINFNGEQMFDVKEAIDTKNHQLDSKLFEYFKEKAFPYLSTKHLGVFPDHVIDMFINGYRLSLTNHGPTPVKEGSKDPRGGIFDAVFTRGDQSKLLTSRHDFKEKNLKEISDLIKKELTEGKALGLSHTYANVRINHVINLWGADFDSNGNLKAIYVTDSDSNASIGMKKYFVGVNSAGKVAISAKEIKEDNIGAQVLGLFTLSTGQDSW

SEQ ID NO: 17 - protein, 290 aa, Artificial sequence
  IgG-degrading enzyme mutant
SVWTKGVTPPANFTQGEDVFHAPYVANQGWYDITKTFNGKDDLLCGAATAGNMLHWWFDQNKDQIKRYLEEHPEKQKINFNGEQMFDVKEAIDTKNHQLDSKLFEYFKEKAFPYLSTKHLGVFPDHVIDMFINGYRLSLTNHGPTPVKEGSKDPRGGIFDAVFTRGDQSKLLTSRHDFKEKNLKEISDLIKKELTEGKALGLSHTYANVRINHVINLWGADFDSNGNLKAIYVTDSDSNASIGMKKYFVGVNSAGKVAISAKEIKEDNIGAQVLGLFTLSTGQDSWNQTN

SEQ ID NO: 18 - protein, 290 aa, Artificial sequence
  IgG-degrading enzyme mutant
SVWTKGVTPPANFTQGEDVFHAPYVANQGWYDITKTFNGKDDLLCGAATAGNMLHWWFDQNKDQIKRYLEEHPEKQKINFKGEQMFDVKEAIDTKNHQLDSKLFEYFKEKAFPYLSTKHLGVFPDHVIDMFINGYRLSLTNHGPTPVKEGSKDPRGGIFDAVFTRGNQSKLLTSRHDFKEKNLKEISDLIKKELTEGKALGLSHTYANVRINHVINLWGADFDSNGNLKAIYVTDSDSNASIGMKKYFVGVNSAGKVAISAKEIKEDNIGAQVLGLFTLSTGQDSWNQTN

SEQ ID NO: 19 - protein, 290 aa, Artificial sequence
  IgG-degrading enzyme mutant
SVWTKGVTPPANFTQGEDVFHAPYVANQGWYDITKTFNGKDDLLCGAATAGNMLHWWFDQNKDQIERYLEEHPEKQKINFKGEQMFDVKKAIDTKNHQLDSKLFEYFKEKAFPYLSTKHLGVFPDHVIDMFINGYRLSLTNHGPTPVKEGSKDPRGGIFDAVFTRGNQSKLLTSRHDFKEKNLKEISDLIKEELTKGKALGLSHTYANVRINHVINLWGADFDSNGNLKAIYVTDSDSNASIGMKKYFVGVNSAGKVAISAKEIKEDNIGAQVLGLFTLSTGQKSWNQTN

SEQ ID NO: 20 - protein, 319 aa, Artificial sequence
  IgG-degrading enzyme mutant
DDYQRNATEAYAKEVPHQITSVWTKGVTPPANFTQGEDVFHAPYVANQGWYDITKTFNGKDDLLCGAATAGNMLHWWFDQNKDQIERYLEEHPEKQKINFKGEQMFDVKKAIDTKNHQLDSKLFEYFKEKAFPYLSTKHLGVFPDHVIDMFINGYRLSLTNHGPTPVKEGSKDPRGGIFDAVFTRGNQSKLLTSRHDFKEKNLKEISDLIKEELTKGKALGLSHTYANVRINHVINLWGADFDSNGNLKAIYVTDSDSNASIGMKKYFVGVNSAGKVAISAKEIKEDNIGAQVLGLFTLSTGQKSWNQTNGGGHHHHHH

SEQ ID NO: 21 - protein, 313 aa, Artificial sequence
  IgG-degrading enzyme mutant
DDYQRNATEAYAKEVPHQITSVWTKGVTPLTPEQFRYNNEDVFHAPYVANQGWYDITKAFDGKDNLLCGAATAGNMLHWWFDQNKDQIKRYLEEHPEKQKINFNGDNMFDVKKAIDTKNHQLDSKLFNYFKEKAFPGLSARRIGVFPDHVIDMFINGYRLSLTNHGPTPVKEGSKDPRGGIFDAVFTRGNQSKLLTSRHDFKNKNLNDISTIIKQELTKGKALGLSHTYANVSINHVINLWGADFNAEGNLEAIYVTDSDSNASIGMKKYFVGVNAHGHVAISAKKIEGENIGAQVLGLFTLSTGQDSWQKLS

SEQ ID NO: 22 - protein, 315 aa, Artificial sequence
  IgG-degrading enzyme mutant
DDYQRNATEAYAKEVPHQITSVWTKGVTPLTPEQFRYNNEDVIHAPYLANQGWYDITKAFDGKDNLLCGAATAGNMLHWWFDQNKTEIEAYLSKHPEKQKIIFRNQELFDLKEAIRTKDSQTNSQLFEYFRDKAFPYLSARQLGVMPDLVLDMFINGYYLNVFKTQSTDVKRPYQDKDKRGGIFDAVFTRGNQTTLLTARHDLKNKGLNDISTIIKEELTKGRALALSHTYANVSISHVINLWGADFNAEGNLEAIYVTDSDANASIGMKKYFVGINKHGHVAISAKKIEGENIGAQVLGLFTLSSGKDIWQKLN

SEQ ID NO: 23 - protein, 315 aa, Artificial sequence
  IgG-degrading enzyme mutant
DDYQRNATEAYAKEVPHQITSVWTKGVTPLTPEQFRYNNEDVIHAPYLAHQGWYDITKTFNGKDNLLCGAATAGNMLHWWFDQNKTEIEAYLSKHPEKQKIIFNNEELFDLKAAIDTKDSQTNSQLFNYFKEKAFPNLSTRQLGVMPDLVLDMFINGYYLNVFKTQSTDVNRPYQDKDKRGGIFDAVFTRGNQTTLLTARHDFKEKGLKDISTIIKQELTEGRALALSHTYANVSISHVINLWGADFDAEGNLKAIYVTDSDANASIGMKKYFVGINAHGKVAISAKKIEGENIGAQVLGLFTLSSGKDIWQQLS

SEQ ID NO: 24 - protein, 315 aa, Artificial sequence
  IgG-degrading enzyme mutant
DSFSANQEIRYSEVTPYHVTSVWTKGVTPLTPEQFRYNNEDVIHAPYLAHQGWYDITKAFDGKDNLLCGAATAGNMLHWWFDQNKTEIEAYLSKHPEKQKIIFNNQELFDLKAAIDTKDSQTNSQLFNYFRDKAFPNLSARQLGVMPDLVLDMFINGYYLNVFKTQSTDVNRPYQDKDKRGGIFDAVFTRGDQTTLLTARHDLKNKGLNDISTIIKQELTEGRALALSHTYANVSISHVINLWGADFNAEGNLEAIYVTDSDANASIGMKKYFVGINAHGHVAISAKKIEGENIGAQVLGLFTLSSGKDIWQKLS

SEQ ID NO: 25 - protein, 295 aa, Artificial sequence
  IgG-degrading enzyme mutant
SVWTKGVTPLTPEQFRYNNEDVIHAPYLAHQGWYDITKAFDGKDNLLCGAATAGNMLHWWFDQNKTEIEAYLSKHPEKQKIIFNNQELFDLKAAIDTKDSQTNSQLFNYFRDKAFPNLSARQLGVMPDLVLDMFINGYYLNVFKTQSTDVNRPYQDKDKRGGIFDAVFTRGDQTTLLTARHDLKNKGLNDISTIIKQELTEGRALALSHTYANVSISHVINLWGADFNAEGNLEAIYVTDSDANASIGMKKYFVGINAHGHVAISAKKIEGENIGAQVLGLFTLSSGKDIWQKLS

SEQ ID NO: 26 - protein, 314 aa, Artificial sequence
  IgG-degrading enzyme mutant
DDYQRNATEAYAKEVPHQITSVWTKGVTPLTPEQFTQGEDVIHAPYLAHQGWYDITKAFDGKDNLLCGAATAGNMLHWWFDQNKTEIEAYLSKHPEKQKIIFNNQELFDLKAAIDTKDSQTNSQLFNYFRDKAFPNLSARQLGVMPDLVLDMFINGYYLNVFKTQSTDVNRPYQDKDKRGGIFDAVFTRGDQTTLLTARHDLKNKGLNDISTIIKQELTEGRALALSHTYANVSISHVINLWGADFNAEGNLEAIYVTDSDANASIGMKKYFVGINAHGHVAISAKKIEGENIGAQVLGLFTLSSGKDIWQKLS

SEQ ID NO: 27 - protein, 312 aa, Artificial sequence
  IgG-degrading enzyme mutant
DDYQRNATEAYAKEVPHQITSVWTKGVTPPEQFTQGEDVIHAPYLAHQGWYDITKAFDGKDNLLCGAATAGNMLHWWFDQNKTEIEAYLSKHPEKQKIIFNNQELFDLKAAIDTKDSQTNSQLFNYFRDKAFPNLSARQLGVMPDLVLDMFINGYYLNVFKTQSTDVNRPYQDKDKRGGIFDAVFTRGDQTTLLTARHDLKNKGLNDISTIIKQELTEGRALALSHTYANVSISHVINLWGADFNAEGNLEAIYVTDSDANASIGMKKYFVGINAHGHVAISAKKIEGENIGAQVLGLFTLSSGKDIWQKLS

SEQ ID NO: 28 - protein, 313 aa, Artificial sequence
  IgG-degrading enzyme mutant
DDYQRNATEAYAKEVPHQITSVWTKGVTPPEQFRYNNEDVIHAPYLAHQGWYDITKAFDGKDNLLCGAATAGNMLHWWFDQNKTEIEAYLSKHPEKQKIIFNNQELFDLKAAIDTKDSQTNSQLFNYFRDKAFPNLSARQLGVMPDLVLDMFINGYYLNVFKTQSTDVNRPYQDKDKRGGIFDAVFTRGDQTTLLTARHDLKNKGLNDISTIIKQELTEGRALALSHTYANVSISHVINLWGADFNAEGNLEAIYVTDSDANASIGMKKYFVGINAHGHVAISAKKIEGENIGAQVLGLFTLSSGKDIWQKLS

SEQ ID NO: 29 - protein, 312 aa, Artificial sequence
  IgG-degrading enzyme mutant
DDYQRNATEAYAKEVPHQITSVWTKGVTPPEQFTQGEDVIHAPYLAHQGWYDITKAFDGKDNLLCGAATAGNMLHWWFDQNKTEIEAYLSKHPEKQKIIINNQELFDLKAAIDTKDSQTNSQLFNYFRDKAFPNLSARQLGVMPDLVLDMFINGYYLNVFKTQSTDVNRPYQDKDKRGGIFDAVFTRGDQTTLLTARHDLKNKGLNDISTIIKQELTEGRALALSHTYANVSISHVINLWGADFNAEGNLEAIYVTDSDANASIGMKKYFVGINAHGHVAISAKKIEGENIGAQVLGLFTLSSGKDIWQKLS

SEQ ID NO: 30 - protein, 312 aa, Artificial sequence
  IgG-degrading enzyme mutant
DDYQRNATEAYAKEVPHQITSVWTKGVTPPEQFTQGEDVIHAPYLAHQGWYDITKAFDGKDNLLCGAATAGNMLHWWFDQNKTEIEAYLSKHPEKQKIIFRNQELFDLKAAIDTKDSQTNSQLFNYFRDKAFPNLSARQLGVMPDLVLDMFINGYYLNVFKTQSTDVNRPYQDKDKRGGIFDAVFTRGDQTTLLTARHDLKNKGLNDISTIIKQELTEGRALALSHTYANVSISHVINLWGADFNAEGNLEAIYVTDSDANASIGMKKYFVGINAHGHVAISAKKIEGENIGAQVLGLFTLSSGKDIWQKLS

SEQ ID NO: 31 - protein, 312 aa, Artificial sequence
  IgG-degrading enzyme mutant
DDYQRNATEAYAKEVPHQITSVWTKGVTPPEQFTQGEDVIHAPYLAHQGWYDITKAFDGKDNLLCGAATAGNMLHWWFDQNKTEIEAYLSKHPEKQKIIIRNQELFDLKAAIDTKDSQTNSQLFNYFRDKAFPNLSARQLGVMPDLVLDMFINGYYLNVFKTQSTDVNRPYQDKDKRGGIFDAVFTRGDQTTLLTARHDLKNKGLNDISTIIKQELTEGRALALSHTYANVSISHVINLWGADFNAEGNLEAIYVTDSDANASIGMKKYFVGINAHGHVAISAKKIEGENIGAQVLGLFTLSSGKDIWQKLS

SEQ ID NO: 32 - protein, 312 aa, Artificial sequence
  IgG-degrading enzyme mutant
DDYQRNATEAYAKEVPHQITSVWTKGVTPPEQFTQGEDVIHAPYLANQGWYDITKAFDGKDNLLCGAATAGNMLHWWFDQNKTEIEAYLSKHPEKQKIIFRNQELFDLKEAIRTKDSQTNSQLFEYFRDKAFPYLSARQLGVMPDLVLDMFINGYYLNVFKTQSTDVKRPYQDKDKRGGIFDAVFTRGNQTTLLTARHDLKNKGLNDISTIIKEELTKGRALALSHTYANVSISHVINLWGADFNAEGNLEAIYVTDSDANASIGMKKYFVGINKHGHVAISAKKIEGENIGAQVLGLFTLSSGKDIWQKLN

SEQ ID NO: 33 - protein, 292 aa, Artificial sequence
  IgG-degrading enzyme mutant
SVWTKGVTPPEQFTQGEDVIHAPYLAHQGWYDITKAFDGKDNLLCGAATAGNMLHWWFDQNKTEIEAYLSKHPEKQKIIFRNQELFDLKAAIDTKDSQTNSQLFNYFRDKAFPNLSARQLGVMPDLVLDMFINGYYLNVFKTQSTDVNRPYQDKDKRGGIFDAVFTRGNQTTLLTARHDLKNKGLNDISTIIKQELTEGRALALSHTYANVSISHVINLWGADFNAEGNLEAIYVTDSDANASIGMKKYFVGINAHGHVAISAKKIEGENIGAQVLGLFTLSSGKDIWQKLS

SEQ ID NO: 34 - protein, 312 aa, Artificial sequence
  IgG-degrading enzyme mutant
DDYQRNATEAYAKEVPHQITSVWTKGVTPPEQFTQGEDVIHAPYLAHQGWYDITKAFDGADNLLCGAATAGNMLHWWFDQNKTEIEAYLSKHPEKQKIIFRNQELFDLKAAIDTKDSQTNSQLFNYFRDKAFPNLSARQLGVMPDLVLDMFINGYYLNVFKTQSTDVNRPYQDKDKRGGIFDAVFTRGNQTTLLTARHDLKNKGLNDISTIIKQELTEGRALALSHTYANVSISHVINLWGADFNAEGNLEAIYVTDSDANASIGMKKYFVGINAHGHVAISAKKIEGENIGAQVLGLFTLSSGKDIWQKLS

SEQ ID NO: 35 - protein, 292 aa, Artificial sequence
  IgG-degrading enzyme mutant
SVWTKGVTPPEQFTQGEDVIHAPYLAHQGWYDITKAFDGADNLLCGAATAGNMLHWWFDQNKTEIEAYLSKHPEKQKIIFRNQELFDLKAAIDTKDSQTNSQLFNYFRDKAFPNLSARQLGVMPDLVLDMFINGYYLNVFKTQSTDVNRPYQDKDKRGGIFDAVFTRGNQTTLLTARHDLKNKGLNDISTIIKQELTEGRALALSHTYANVSISHVINLWGADFNAEGNLEAIYVTDSDANASIGMKKYFVGINAHGHVAISAKKIEGENIGAQVLGLFTLSSGKDIWQKLS

SEQ ID NO: 36 - protein, 312 aa, Artificial sequence
  IgG-degrading enzyme mutant
DDYQRNATEAYAKEVPHQITSVWTKGVTPPEQFTQGEDVIHAPYLAHQGWYDITKAFDGKDNLLCGAATAGNMLHWWFDQNKTEIEAYLSKHPEKQKIIFRNQELFDLKAAIDTKDSQTNSQLFNYFRDKAFPNLSARQLGVMPDLVLDMFINGYYLNVFKTQSTDVNRPYQDKDKRGGIFDAVFTRGNQTTLLTARHDLKNKGLNDISTIIKQELTEGRALALSHTYANVSISHVINLWGADFNAEGNLEAIYVTDSDANASIGMKKYFVGINAHGHVAISAKKIEGENIGAQVLGLFTLSSGKDIWQKLS

SEQ ID NO: 37 - protein, 312 aa, Artificial sequence
  IgG-degrading enzyme mutant
DDYQRNATEAYAKEVPHQITSVWTKGVTPLTPEQFTQGEDVFHAPYVANQGWYDITKAFDGKDNLLCGAATAGNMLHWWFDQNKDQIKRYLEEHPEKQKINFNGENMFDVKKAIDTKNHQLDSKLFNYFKEKAFPYLSAKHLGVFPDHVIDMFINGYRLSLTNHGPTPVKEGSKDPRGGIFDAVFTRGNQSKLLTSRHDFKNKNLNDISTIIKQELTKGKALGLSHTYANVRINHVINLWGADFNAEGNLEAIYVTDSDSNASIGMKKYFVGVNAHGHVAISAKKIEGENIGAQVLGLFTLSTGQDSWQKLS

SEQ ID NO: 38 - protein, 312 aa, Artificial sequence
  IgG-degrading enzyme mutant
DDYQRNATEAYAKEVPHQITSVWTKGVTPLTPEQFTQGEDVFHAPYVANQGWYDITKAFDGKDNLLCGAATAGNMLHWWFDQNKDQIKRYLEEHPEKQKINFRGENMFDVKEAIRTKNHQLDSKLFEYFKEKAFPYLSAKHLGVFPDHVIDMFINGYRLSLTNHGPTPVKKGSKDPRGGIFDAVFTRGNQSKLLTSRHDFKNKNLNDISTIIKSELTNGKALGLSHTYANVRINHVINLWGADFNAEGNLEAIYVTDSDSNASIGMKKYFVGVNKHGHVAISAKKIEGENIGAQVLGLFTLSTGQDSWQKLN

SEQ ID NO: 39 - protein, 312 aa, Artificial sequence
  IgG-degrading enzyme mutant
DDYQRNATEAYAKEVPHQITSVWTKGVTPLTPEQFTQGEDVFHAPYVANQGWYDITKTFNGKDDLLCGAATAGNMLHWWFDQNKDQIKRYLEEHPEKQKINFNGEQMFDVKEAIDTKNHQLDSKLFEYFKEKAFPYLSTKHLGVFPDHVIDMFINGYRLSLTNHGPTPVKEGSKDPRGGIFDAVFTRGNQSKLLTSRHDFKEKNLKEISDLIKQELTEGKALGLSHTYANVRINHVINLWGADFDAEGNLKAIYVTDSDSNASIGMKKYFVGVNAAGKVAISAKKIEGENIGAQVLGLFTLSTGQDSWNQTS

SEQ ID NO: 40 - protein, 312 aa, Artificial sequence
  IgG-degrading enzyme mutant
DDYQRNATEAYAKEVPHQITSVWTKGVTPLTPEQFTQGEDVFHAPYVANQGWYDITKTFNGKDDLLCGAATAGNMLHWWFDQNKDQIKRYLEEHPEKQKINFRGEQMFDVKEAIRTKNHQLDSKLFEYFKEKAFPYLSTKHLGVFPDHVIDMFINGYRLSLTNHGPTPVKKGSKDPRGGIFDAVFTRGNQSKLLTSRHDFKEKNLKEISDLIKEELTKGKALGLSHTYANVRINHVINLWGADFDAEGNLKAIYVTDSDSNASIGMKKYFVGVNKAGKVAISAKKIEGENIGAQVLGLFTLSTGQDSWNQTN

SEQ ID NO: 41 - protein, 310 aa, Artificial sequence
  IgG-degrading enzyme mutant
DDYQRNATEAYAKEVPHQITSVWTKGVTPPEQFTQGEDVIHAPYVANQGWYDITKAFDGKDNLLCGAATAGNMLHWWFDQNKDQIKRYLEEHPEKQKINFRGEQMFDVKKAIDTKNHQLDSKLFNYFKEKAFPGLSARRIGVFPDHVIDMFINGYRLSLTNHGPTPVKEGSKDPRGGIFDAVFTRGNQSKLLTSRHDFKNKNLNDISTIIKQELTKGKALGLSHTYANVSINHVINLWGADFNAEGNLEAIYVTDSDSNASIGMKKYFVGVNAHGHVAISAKKIEGENIGAQVLGLFTLSTGQDSWQKLS

SEQ ID NO: 42 - protein, 995 aa, Artificial sequence
  EndoS
MDKHLLVKRTLGCVCAATLMGAALATHHDSLNTVKAEEKTVQVQKGLPSIDSLHYLSENSKKEFKEELSKAGQESQKVKEILAKAQQADKQAQELAKMKIPEKIPMKPLHGPLYGGYFRTWHDKTSDPTEKDKVNSMGELPKEVDLAFIFHDWTKDYSLFWKELATKHVPKLNKQGTRVIRTIPWRFLAGGDNSGIAEDTSKYPNTPEGNKALAKAIVDEYVYKYNLDGLDVDVEHDSIPKVDKKEDTAGVERSIQVFEEIGKLIGPKGVDKSRLFIMDSTYMADKNPLIERGAPYINLLLVQVYGSQGEKGGWEPVSNRPEKTMEERWQGYSKYIRPEQYMIGFSFYEENAQEGNLWYDINSRKDEDKANGINTDITGTRAERYARWQPKTGGVKGGIFSYAIDRDGVAHQPKKYAKQKEFKDATDNIFHSDYSVSKALKTVMLKDKSYDLIDEKDFPDKALREAVMAQVGTRKGDLERFNGTLRLDNPAIQSLEGLNKFKKLAQLDLIGLSRITKLDRSVLPANMKPGKDTLETVLETYKKDNKEEPATIPPVSLKVSGLTGLKELDLSGFDRETLAGLDAATLTSLEKVDISGNKLDLAPGTENRQIFDTMLSTISNHVGSNEQTVKFDKQKPTGHYPDTYGKTSLRLPVANEKVDLQSQLLFGTVTNQGTLINSEADYKAYQNHKIAGRSFVDSNYHYNNFKVSYENYTVKVTDSTLGTTTDKTLATDKEETYKVDFFSPADKTKAVHTAKVIVGDEKTMMVNLAEGATVIGGSADPVNARKVFDGQLGSETDNISLGWDSKQSIIFKLKEDGLIKHWRFFNDSARNPETTNKPIQEASLQIFNIKDYNLDNLLENPNKFDDEKYWITVDTYSAQGERATAFSNTLNNITSKYWRVVFDTKGDRYSSPVVPELQILGYPLPNADTIMKTVTTAKELSQQKDKFSQKMLDELKIKEMALETSLNSKIFDVTAINANAGVLKDCIEKRQLLKK

SEQ ID NO: 43 - protein, 335 aa, Artificial sequence
  EndoF2
MKTANFSFALCLSVVIMLFIKCTRSEQDLSVTKDAIAQKSGVTVSAVNLSNLIAYKNSDHQISAGYYRTWRDSATASGNLPSMRWLPDSLDMVMVFPDYTPPENAYWNTLKTNYVPYLHKRGTKVIITLGDLNSATTTGGQDSIGYSSWAKGIYDKWVGEYNLDGIDIDIESSPSGATLTKFVAATKALSKYFGPKSGTGKTFVYDTNQNPTNFFIQTAPRYNYVFLQAYGRSTTNLTTVSGLYAPYISMKQFLPGFSFYEENGYPGNYWNDVRYPQNGTGRAYDYARWQPATGKKGGVFSYAIERDAPLTSSNDNTLRAPNFRVTKDLIKIMNP

SEQ ID NO: 44 - protein, 837 aa, Artificial sequence
  EndoE
MNGVQKGMVFKVGNNLSTRKGENRETIVSWLGLSLLVGLAFILFSLFHQPMISQANEPTQEKHFMVYYRAWRDKTMQGVNTTLPDENWLTMHDIPYGIDIVNVFSYVPKGQEALAQPFYDTLKNEYAPALHARGVRLVRGIDYSELLKVPYAGTTPTEAEFDAYAKELLTKFVDDLGIDGLDIDMETRPSEKDIVLSNGVIRALSKYIGPKSGTDRPFLYDTNAEYLPPLQDVSDCFDFLAYQQYGSDDQRTQRALNNLSPVLNGERFVPGLTFPEEQDRNRWYDTKEPYMESNMYKVARYSYENNLGGMFLYALDRDGRTYNEDDLNQIKPSNLLWTKTAIAESKGVSLAEMKAAAQHYLKRISYANTDLEAQNKAAEAVTQATTLYDVNKAILGGDYGQGLSNTYDAELEKGLLAIDLTTLYRALDQAVAAIEKAESYTPETIQALQTTKESVATELAGKTYTAAQVTTWQTEVQTALDNLKEKQTQPLKSVFSIDAGRKYFSVEQLEELVAKASQNGYTDVQLILGNDGLRFILDDMSVNVNGKKYNHNRVSKAIQRGNNAYYNDPNGNALTQKEMDRLLAFAKARNINIIPVINSPGHMDALLVAMEKLAIKNPAFDGSKRPVDLGNQKAVNFTKAIISKYVAYFSAHSEIFNFGGDEYANDVDTGGWAKLQSSGRYKDFVAYANDLAKIIKDAGMQPMSFNDGIYYNSDDSFGTFDPEIIISYWTAGWSGYDVAKPEYFVQKGHKIFNTNDAWYWVAGNVDSGIYQYDDALANMSKKAFTDVPAGSPNLPIIGSIQCVWYDDPRRDYDFERIYTLMDTFSENYREYMVVKNH

SEQ ID NO: 45 - protein, 379 aa, Artificial sequence
  CP40
MHNSPRSVSRLITVGITSALFASTFSAVASAESATLSKEPLKASPGRADTVGVQTTCNAKPIFFGYYRTWRDKAIQLKDDDPWKDKLQVKLTDIPEHVNMVSLFHVEDNQKSDQQFWETFHREYQPELKKRGTRVVRTVGAQLLLNKIKDKNLYGKHVEDDYKYREIARDVYNEYVVKHNLDGLDVDMELRQVEKQLNLKWQLRKIMGAFSELMGPKAPANEGKKPDHEGYKYLIYDTFDNAQTSQVGLVADLVDYVLAQTYKKDTKESVTQVWNGFRDKINSCQFMAGYAHPEENDTNRFLTAVGEVNKSGAMQVAEWKPEGGEKGGTFAYALDRDGRTYDGDDFTTLKPTDFAFTKRAIELTTGESSTDLGKPTGSR

SEQ ID NO: 46 - DNA, 957 bp, Artificial sequence
  IdeS
gatagctttagcgcaaaccaggagatccgctatagcgaggttaccccgtatcacgttaccagcgtttggaccaaaggcgttaccccgccggccaactttacccagggcgaagacgtgtttcatgccccgtatgttgccaatcagggctggtacgacatcaccaaaaccttcaatggcaaggacgatctgctgtgcggtgccgcaaccgccggtaacatgctgcactggtggttcgaccagaataaagaccagatcaaacgctacctggaggaacacccggaaaaacagaaaattaatttcaacggcgaacagatgtttgatgtgaaagaagctattgataccaagaaccaccagctggacagcaagctgttcgaatattttaaggagaaagccttcccgtacctgagcaccaaacatctgggcgtgtttccggaccatgtgatcgacatgttcatcaacggctatcgcctgagcctgaccaatcatggtccgaccccggtgaaagaaggtagcaaagatccgcgcggtggtatcttcgatgccgtgtttacacgtggcgatcagagtaagctgctgaccagccgccatgattttaaagagaaaaatctgaaagaaatcagcgatctgattaagaaggagctgaccgagggcaaagccctgggcctgagccacacctacgccaatgtgcgcatcaaccacgtgatcaacctgtggggtgccgactttgatagcaacggcaacctgaaggcaatttacgtgaccgacagcgacagcaatgccagtattggcatgaaaaaatactttgttggtgtgaacagcgccggcaaagtggcaatcagtgccaaggagatcaaagaagataacatcggcgcccaggttctgggtctgtttaccctgagcacaggtcaggatagctggaatcagaccaatcatcatcaccaccatcacagtagtggt

SEQ ID NO: 47 - DNA, 963 bp, Artificial sequence
  IdeE
gatgactatcaaagaaacgcgacggaggcctatgctaaggaggtccctcatcaaattacgtccgtttggactaagggggttaccccactgactcccgagcagtttagatataataacgaagatgtcatccatgccccataccttgcgcaccagggttggtacgacataacaaaggcttttgacggcaaagataaccttctgtgtggtgcggcaactgccggtaacatgcttcattggtggttcgatcaaaacaaaacagaaattgaggcgtaccttagtaaacaccccgaaaaacagaagatcatcttcaacaaccaggagctttttgacttaaaggccgctattgatacgaaggatagtcagacgaacagtcaattatttaactatttcagagacaaagcgttcccaaaccttagcgcgcgccaactgggcgttatgcctgacctggtgttggacatgttcattaacggatattacctgaatgtatttaaaactcaatcgactgatgtcaaccgcccttaccaggacaaggataaacgtggtggcatatttgacgcagtatttacacgtggggaccaaacgacacttttaactgcgcggcacgaccttaaaaacaagggtctgaatgatatctcaactataattaagcaggaacttactgagggacgcgcattggctttgtcacatacttacgcaaacgtatctatttcccatgtgattaacttgtggggggccgattttaacgctgagggaaatctggaagctatctatgtgactgactccgacgctaacgcttcaatcgggatgaagaaatacttcgtgggaataaacgcccaccgccacgttgcgataagcgccaaaaagatagagggggaaaacataggcgcacaggtattggggttgtttacactgtcatcgggaaaggatatttggcaaaagctgtcgcatcaccatcatcaccac